European Patent Application EP 4 644 415 A1, published November 5, 2025. Title: ANTI-FIBRIN AGENT. Applicant: SYNAPSE B.V. The sequence listing filed with the application follows.

SEQUENCE LISTING (39 sequences)

SEQ ID NO: 1 - protein, 8 aa, synthetic construct
GTSFDINT

SEQ ID NO: 2 - protein, 8 aa, synthetic construct
GTILDINT

SEQ ID NO: 3 - protein, 8 aa, synthetic construct
GSIFSINA

SEQ ID NO: 4 - protein, 8 aa, synthetic construct
GRTFSTAT

SEQ ID NO: 5 - protein, 7 aa, synthetic construct
NTEGITN

SEQ ID NO: 6 - protein, 7 aa, synthetic construct
TSAGITD

SEQ ID NO: 7 - protein, 7 aa, synthetic construct
TSGGSTN

SEQ ID NO: 8 - protein, 11 aa, synthetic construct
TVTGGVTRSAL

SEQ ID NO: 9 - protein, 14 aa, synthetic construct
NAWIRGINRLYDNY

SEQ ID NO: 10 - protein, 14 aa, synthetic construct
NAWVRGTNRLYDNY

SEQ ID NO: 11 - protein, 14 aa, synthetic construct
NVNYYNDYGVPYDY

SEQ ID NO: 12 - protein, 17 aa, synthetic construct
AAVGRLGVFARANEYDY

SEQ ID NO: 13 - protein, 25 aa, synthetic construct [sequence omitted]

SEQ ID NO: 14 - protein, 25 aa, synthetic construct
EVQLVESGGGLVQAGGSLRLSCAAS

SEQ ID NO: 15 - protein, 19 aa, synthetic construct
MTTWYRQAPGAQRELVATI

SEQ ID NO: 16 - protein, 17 aa, synthetic construct
MTWYRQPGAQRELVATI

SEQ ID NO: 17 - protein, 18 aa, synthetic construct
MGWYRQAPGKQRELVAAI

SEQ ID NO: 18 - protein, 18 aa, synthetic construct
MGWFRQAPGKEREFVARI

SEQ ID NO: 19 - protein, 37 aa, synthetic construct
YADFVEGRFTISRDNAKNTVYLQMNNLKPEDTAVYYC

SEQ ID NO: 20 - protein, 37 aa, synthetic construct
YADFVKGRFAISRDNTKNTVYLQMNNLKPEDTAVYYC

SEQ ID NO: 21 - protein, 37 aa, synthetic construct
YADSVKGRFTISRDNAKSTVYLQMYSLKPEDTAVYFC

SEQ ID NO: 22 - protein, 37 aa, synthetic construct
YGDPVKGRFTISRDNAKNTVYLQMANLKPEDTAVYYC

SEQ ID NO: 23 - protein, 11 aa, synthetic construct
WGQGTQVTVSS

SEQ ID NO: 24 - protein, 11 aa, synthetic construct
WGQGTRVTVSS

SEQ ID NO: 25 - protein, 121 aa, Lama glama
EVQLVESGGGLVQPGGSLRLSCAASGTSFDINTMTTWYRQAPGAQRELVATINTEGITNYADFVEGRFTISRDNAKNTVYLQMNNLKPEDTAVYYCNAWIRGINRLYDNYWGQGTQVTVSS

SEQ ID NO: 26 - protein, 119 aa, synthetic construct
EVQLVESGGGLVQPGGSLRLSCAASGTILDINTMTWYRQPGAQRELVATITSAGITDYADFVKGRFAISRDNTKNTVYLQMNNLKPEDTAVYYCNAWVRGTNRLYDNYWGQGTQVTVSS

SEQ ID NO: 27 - protein, 120 aa, synthetic construct
EVQLVESGGGLVQPGGSLRLSCAASGSIFSINAMGWYRQAPGKQRELVAAITSGGSTNYADSVKGRFTISRDNAKSTVYLQMYSLKPEDTAVYFCNVNYYNDYGVPYDYWGQGTRVTVSS

SEQ ID NO: 28 - protein, 127 aa, synthetic construct
EVQLVESGGGLVQAGGSLRLSCAASGRTFSTATMGWFRQAPGKEREFVARITVTGGVTRSALYGDPVKGRFTISRDNAKNTVYLQMANLKPEDTAVYYCAAVGRLGVFARANEYDYWGQGTQVTVSS

SEQ ID NO: 29 - protein, 276 aa, Homo sapiens
KPSSPPEELKFQCGQKTLRPRFKIIGGEFTTIENQPWFAAIYRRHRGGSVTYVCGGSLMSPCWVISATHCFIDYPKKEDYIVYLGRSRLNSNTQGEMKFEVENLILHKDYSADTLAHHNDIALLKIRSKEGRCAQPSRTIQTICLPSMYNDPQFGTSCEITGFGKENSTDYLYPEQLKMTVVKLISHRECQQPHYYGSEVTTKMLCAADPQWKTDSCQGDSGGPLVCSLQGRMTLTGIVSWGRGCALKDKPGVYTRVSHFLPWIRSHTKEENGLAL

SEQ ID NO: 30 - protein, 6 aa, unidentified
SSSGSG

SEQ ID NO: 31 - protein, 128 aa, synthetic construct
EVQLVESGGGLVQXGGSLRLSCAASGXXXXXXXMXXWXRXXPGXXREXVAXIXXXGXXXXXXXYXDXVXGRFXISRDNXKXTVYLQMXXLKPEDTAVYXCXXXXXXXXXXXXXXXXYWGQGTXVTVSS

SEQ ID NO: 32 - protein, 34 aa, Homo sapiens
GPRVVERHQSACKDSDWPFCSDEDWNYKCPSGCR

SEQ ID NO: 33 - protein, 7 aa, Homo sapiens
WPFCSDE

SEQ ID NO: 34 - protein, 847 aa, Homo sapiens
ADSGEGDFLAEGGGVRGPRVVERHQSACKDSDWPFCSDEDWNYKCPSGCRMKGLIDEVNQDFTNRINKLKNSLFEYQKNNKDSHSLTTNIMEILRGDFSSANNRDNTYNRVSEDLRSRIEVLKRKVIEKVQHIQLLQKNVRAQLVDMKRLEVDIDIKIRSCRGSCSRALAREVDLKDYEDQQKQLEQVIAKDLLPSRDRQHLPLIKMKPVPDLVPGNFKSQLQKVPPEWKALTDMPQMRMELERPGGNEITRGGSTSYGTGSETESPRNPSSAGSWNSGSSGPGSTGNRNPGSSGTGGTATWKPGSSGPGSTGSWNSGSSGTGSTGNQNPGSPRPGSTGTWNPGSSERGSAGHWTSESSVSGSTGQWHSESGSFRPDSPGSGNARPNNPDWGTFEEVSGNVSPGTRREYHTEKLVTSKGDKELRTGKEKVTSGSTTTTRRSCSKTVTKTVIGPDGHKEVTKEVVTSEDGSDCPEAMDLGTLSGIGTLDGFRHRHPDEAAFFDTASTGKTFPGFFSPMLGEFVSETESRGSESGIFTNTKESSSHHPGIAEFPSRGKSSSYSKQFTSSTSYNRGDSTFESKSYKMADEAGSEADHEGTHSTKRGHAKSRPVRDCDDVLQTHPSGTQSGIFNIKLPGSSKIFSVYCDQETSLGGWLLIQQRMDGSLNFNRTWQDYKRGFGSLNDEGEGEFWLGNDYLHLLTQRGSVLRVELEDWAGNEAYAEYHFRVGSEAEGYALQVSSYEGTAGDALIEGSVEEGAEYTSHNNMQFSTFDRDADQWEENCAEVYGGGWWYNNCQAANLNGIYYPGGSYDPRNNSPYEIENGVVWVSFRGADYSLRAVRMKIRPLVTQ

SEQ ID NO: 35 - protein, 7 aa, Homo sapiens
WPFCSDE

SEQ ID NO: 36 - protein, 60 aa, Homo sapiens
ADSGEGDFLAEGGGVRGPRVVERHQSACKDSDWPFCSDEDWNYKCPSGCRMKGLIDEVNQ

SEQ ID NO: 37 - protein, 15 aa, synthetic construct
GGGGSGGGGSGGGGS

SEQ ID NO: 38 - protein, 15 aa, synthetic construct
EAAAKEAAAKEAAAK

SEQ ID NO: 39 - protein, 5 aa, synthetic construct
PAPAP